European Patent Application EP 4 471 141 A1, published December 4, 2024. Title: Nucleic acid molecule capable of blocking motor protein, and construction method and application thereof. Applicant: BGI SHENZHEN. The sequence listing filed with the application follows.

SEQUENCE LISTING (13 sequences)

SEQ ID NO: 1 - DNA, 68 bp, Artificial Sequence
  primer
ttttttttttttttttttttttttttttttttttttttttggttgtttctgttggtgctgatattgct

SEQ ID NO: 2 - DNA, 45 bp, Artificial Sequence
  primer
gcaatatcagcaccaacagaaacaacctttgaggcgagcggtcaa

SEQ ID NO: 3 - DNA, 1320 bp, Artificial Sequence
  Nucleotide sequence of helicase Dda
atgacatttgatgatttgaccgaaggccagaaaaatgcctttaacattgttatgaaggctattaaagaaaagaaacatcatgtaactattaatggacctgctggtaccggtaagactactcttactaagttcatcattgaagctttaatatctacgggtggaactggtattattttagcagctcctacacatgcagctaaaaagattctttcaaaactatcagggaaagaagcgagtactattcatagtattcttaaaattaacccagtaacatatgaagaaaatgttctttttgaacaaaaagaagtacctgatttagccaaatgcagagtattaatctgcgacgaagtgtcaatgtatgatagaaagctatttaaaattctgctttcaactattccaccttggtgtactataattggaataggggataataagcaaatcagacctgttgaaccaggagaaaatactgcttatatcagtccattctttacacataaagatttttatcagtgtgaactcactgaagttaaacgcagtaatgctcctattattgatgtagctactgacgttcgcaacggtaagtggaattatgataaagttgttgacgggcatggagtacgtggatttactggtgataccgctttacgcgattttatggtaaattatttttcaatcgtcaaatcactagatgatttgtttgaaaatcgcgtaatggcatttacgaataaatctgttgacaagttaaatagcattattcgtaaaaagatttttgaaactgataaagattttattgtcggtgaaattattgtaatgcaggaaccattatttaaaacatataaaattgatggaaagcctgtgtcagaaattatttttaataacggacaattagttcgtattatagaagcagagtatacatcaacgtttgttaaagcccgtggtgttcctggagaatatctaattcgtcattgggatttaacagtagaaacttatggcgatgatgaatattatcgtgaaaagattaaaataatttcatctgacgaagaattgtataagtttaacctatttttagctaaaacagcagaaacttataaaaattggaacaaaggcggaaaagctccgtggagtgatttttgggatgctaaatcacagtttagtaaagtgaaagcacttcctgcatcaacattccataaagcgcagggtatgtctgtagaccgtgctttcatttatacgccttgtattcattatgcagatgttgaattagctcaacaacttctttatgttggtgtcacccgtggtcgttatgatgtgttttatgtatga

SEQ ID NO: 4 - protein, 439 aa, Artificial Sequence
  Amino acid sequence of helicase Dda protein
MTFDDLTEGQKNAFNIVMKAIKEKKHHVTINGPAGTGKTTLTKFIIEALISTGGTGIILAAPTHAAKKILSKLSGKEASTIHSILKINPVTYEENVLFEQKEVPDLAKCRVLICDEVSMYDRKLFKILLSTIPPWCTIIGIGDNKQIRPVEPGENTAYISPFFTHKDFYQCELTEVKRSNAPIIDVATDVRNGKWNYDKVVDGHGVRGFTGDTALRDFMVNYFSIVKSLDDLFENRVMAFTNKSVDKLNSIIRKKIFETDKDFIVGEIIVMQEPLFKTYKIDGKPVSEIIFNNGQLVRIIEAEYTSTFVKARGVPGEYLIRHWDLTVETYGDDEYYREKIKIISSDEELYKFNLFLAKTAETYKNWNKGGKAPWSDFWDAKSQFSKVKALPASTFHKAQGMSVDRAFIYTPCIHYADVELAQQLLYVGVTRGRYDVFYV

SEQ ID NO: 5 - DNA, 2045 bp, Artificial Sequence
  pUC57 plasmid digestion product
cgacgctcaagtcagaggtggcgaaacccgacaggactataaagataccaggcgtttccccctggaagctccctcgtgcgctctcctgttccgaccctgccgcttaccggatacctgtccgcctttctcccttcgggaagcgtggcgctttctcatagctcacgctgtaggtatctcagttcggtgtaggtcgttcgctccaagctgggctgtgtgcacgaaccccccgttcagcccgaccgctgcgccttatccggtaactatcgtcttgagtccaacccggtaagacacgacttatcgccactggcagcagccactggtaacaggattagcagagcgaggtatgtaggcggtgctacagagttcttgaagtggtggcctaactacggctacactagaagaacagtatttggtatctgcgctctgctgaagccagttaccttcggaaaaagagttggtagctcttgatccggcaaacaaaccaccgctggtagcggtggtttttttgtttgcaagcagcagattacgcgcagaaaaaaaggatctcaagaagatcctttgatcttttctacggggtctgacgctcagtggaacgaaaactcacgttaagggattttggtcatgagattatcaaaaaggatcttcacctagatccttttaaattaaaaatgaagttttaaatcaatctaaagtatatatgagtaaacttggtctgacagttaccaatgcttaatcagtgaggcacctatctcagcgatctgtctatttcgttcatccatagttgcctgactccccgtcgtgtagataactacgatacgggagggcttaccatctggccccagtgctgcaatgataccgcgagacccacgctcaccggctccagatttatcagcaataaaccagccagccggaagggccgagcgcagaagtggtcctgcaactttatccgcctccatccagtctattaattgttgccgggaagctagagtaagtagttcgccagttaatagtttgcgcaacgttgttgccattgctacaggcatcgtggtgtcacgctcgtcgtttggtatggcttcattcagctccggttcccaacgatcaaggcgagttacatgatcccccatgttgtgcaaaaaagcggttagctccttcggtcctccgatcgttgtcagaagtaagttggccgcagtgttatcactcatggttatggcagcactgcataattctcttactgtcatgccatccgtaagatgcttttctgtgactggtgagtactcaaccaagtcattctgagaatagtgtatgcggcgaccgagttgctcttgcccggcgtcaatacgggataataccgcgccacatagcagaactttaaaagtgctcatcattggaaaacgttcttcggggcgaaaactctcaaggatcttaccgctgttgagatccagttcgatgtaacccactcgtgcacccaactgatcttcagcatcttttactttcaccagcgtttctgggtgagcaaaaacaggaaggcaaaatgccgcaaaaaagggaataagggcgacacggaaatgttgaatactcatactcttcctttttcaatattattgaagcatttatcagggttattgtctcatgagcggatacatatttgaatgtatttagaaaaataaacaaataggggttccgcgcacatttccccgaaaagtgccacctgacgtctaagaaaccattattatcatgacattaacctataaaaataggcgtatcacgaggccctttcgtctcgcgcgtttcggtgatgacggtgaaaacctctgacacatgcagctcccggagacggtcacagcttgtctgtaagcggatgccgggagcagacaagcccgtcagggcgcgtcagcgggtgttggcgggtgtcggggctggcttaactatgcggcatcagagcagattgtactgagagtgcaccatatgcggtgtgaaataccgcacagatgcgtaaggagaaaataccgcatcaggcgccattcgccattcaggctgcgcaactg

SEQ ID NO: 6 - DNA, 2017 bp, Artificial Sequence
  Read sequence
acgcagttgcgcagcgaatggcgaatggcgcctgatgcggtattttctccgccgcatctgtgcggtatttcaccaccgcatgccgttgcactcggtaatctgctcctgatgccacataagattagccagccaccagacaccgccaacacccgctgacgcgccagccgaagcttgtctgctcggcatccgcttacagacaagctgtgaccgtctccgggagctgcatgtgtcagggttttccaccgtcatcaccgaaacgcgcgagacgaagggcctcgtgatgcgcctattttatagtttaatgtcatgataataatggtttcttagacgtcaggtggcacttttccaggaagtagcgcggaacatatttgtttatttttctattgttcaaatatgtatcgctcgcggaataataacccctgataaatgctttaatattgaaaaaggaaagtatggtattcaacatttccgtgtcgcccttattcccttttttgcggcattttgccttctatttttttgctcacccagaaacgctggtgaaaagtaaaagatgctgaagatcagttggggtgcacggagtgagttacatccagactggatctcaacagcgataagatcagcagagagttttcgccccgaagaacgttttccaatgatgagcacttttaaagttctgctggcgcggtatcccgtattgacgccgggcgagcaactcggtcgccgccactattcactgggacgacccggttgagtactcaccagtcacagaaaagcatcttacggatggcagcagcaatgaaattatgcagtgctgccacttaaccatgagtgataacactgcgaccaacacttctgacaacgatcggaggaccgaagagctaaccgctttttgcacaacatggggatcgtaactcgccttgatcgttgggaaccggagctgatgaagccatgcaagcgacaggcgtgacaccacgatgcctgtaacaatggcaacaacgttgcgcaaactattaactggcgaactacttactctgcttccggcaacaattaataaagactggatggcgagataaagttgcaggaccacttctgcatcgacgcttcaagctggctggtttgtgctgataaatctggagccggtgagcgtgggtgcctaacggtatcattgcaactggggccagatggtagccctcacgtatcgtgattgtctacacgacggggagtcgagcaactatggatgaacgaaatagacagatcccgctgaataggtgcctcactgattaaagcattgtcagaccaagtttactccttatatactttagattgatttacttcatttttaatttaaaaaggatctagtgaagatccttttttgataatctcttgaagccaaaatcacttaacgtggtttttcgttccgcactgagcgtcgaggcccgtgaaaaagatcaagaaaagggatgatcttcttgagagatctttttctgcgtaatctgctgcttgcaaagcaaaaaaaccaccgctaccagcggtggtttgttttgccagatcaaaaaactaccaactctttttccgaaggtaaccagcttcagcagagcgcagataccaaatactgttcttcacaaattgtagccgtagttaggcttctgcttcaagaactctgctgcgctaccgcctacatacctcgctactgctaatcctgttaccagtggctgctgccagtggcagtaaatcgtgtcttaccgggttggactcaagacgatagttaccggataaggcgcagcggtcaggctgaacagggggttcgtgcagcccagcttggagcgaacacgaccaccaccgaactgagatacctacagcgtgagcgctatgaaagcgccacgcttcccgaaggagaaaggcggacaggtatccggtaagcggcagggtcggaacaggagagcgcaccagggagcttccaggaaacgcctggtatctttatagtcctgtcgggtttcgccacctctgacgagcgtcg

SEQ ID NO: 7 - DNA, 67 bp, Artificial Sequence
  primer
cgttatagtcgtggttgtctttgttggtttttttttttttttttttttttttttttttttttttttt

SEQ ID NO: 8 - DNA, 46 bp, Artificial Sequence
  primer
aactggcgagcggagtttccaacaaagacaaccacgactataacgt

SEQ ID NO: 9 - DNA, 59 bp, Artificial Sequence
  primer
gtgtttgttagtcgctttttttttttggaattttttttttggaattttttttttgcgct

SEQ ID NO: 10 - DNA, 59 bp, Artificial Sequence
  primer
agcgcaaaaaaaaaattccaaaaaaaaaattccaaaaaaaaaaagcgactaacaaacac

SEQ ID NO: 11 - DNA, 58 bp, Artificial Sequence
  Read sequence
gttctttgcttactcgctttttttttggaatttttttttttggaatttttttttgcgg

SEQ ID NO: 12 - protein, 673 aa, Artificial Sequence
  Amino acid sequence of helicase Rep-X
MRLNPGQQQAVEFVTGPLLVLAGAGSGKTRVITNKIAHLIRGSGYQARHIAAVTFTNKAAREMKERVGQTLGRKEARGLMISTFHTLGLDIIKREYAALGMKANFSLFDDTDQLALLKELTEGLIEDDKVLLQQLISTISNWKNDLKTPSQAAASAIGERDRIFAHVYGLYDAHLKACNVLDFDDLILLPTLLLQRNEEVRKRWQNKIRYLLVDEYQDTNTSQYELVKLLVGSRARFTVVGDDDQSIYSWRGARPQNLVLLSQDFPALKVIKLEQNYRSSGRILKAANILIANNPHVFEKRLFSELGYGAELKVLSANNEEHEAERVTGELIAHHFVNKTQYKDYAILYRGNHQSRVFEKFLMQNRIPYKISGGTSFFSRPEIKDLLAYLRVLTNPDDDCAFLRIVNTPKREIGPATLKKLGEWAMTRNKSMFTASFDMGLSQTLSGRGYEALTRFTHWLAEIQRLAEREPIAAVRDLIHGMDYESWLYETSPSPKAAEMRMKNVNQLFSWMTEMLEGSELDEPMTLTQVVTRFTLRDMMERGESEEELDQVQLMTLHASKGLEFPYVYMVGMEEGFLPHQSSIDEDNIDEERRLAYVGITRAQKELTFTLAKERRQYGELVRPEPSRFLLELPQDDLIWEQERKVVSAEERMQKGQSHLANLKAMMAAKRGK

SEQ ID NO: 13 - protein, 773 aa, Artificial Sequence
  Amino acid sequence of polymerase mutant PGV2
MILDTDYITEDGKPVIRIFKKENGEFKIDYDRNFEPYIYALLKDDSAIEDVKKITAERHGTTVRVVRAEKVKKKFLGRPIEVWKLYFTHPQDQPAIRDKIKEHPAVVDIYEYDIPFAKRYLIDKGLIPMEGDEELKMLAFAIATLYHEGEEFAEGPILMISYADEEGARVITWKNIDLPYVDVVSTEKEMIKRFLKVVKEKDPDVLITYNGDNFDFAYLKKRSEKLGVKFILGREGSEPKIQRMGDRFAVEVKGRIHFDLYPVIRRTINLPTYTLEAVYEAIFGQPKEKVYAEEIAQAWETGEGLERVARYSMEDAKVTYELGKEFFPMEAQLSRLVGQSLWDVSRSSTGNLVEWFLLRKAYERNELAPNKPDERELARRRESYAGGYVKEPERGLWENIVYLDFRSLYPSIIITHNVSPDTLNREGCGEYDVAPQVGHKFCKDFPGFIPSLLGPLLEERQKVKKKMKATIDPIEKKLLDYRQRLIGILANSFYGYYGYAKARWYCKECAESVTAWGRQYLETTIREIEEKFGFKVLYADTDGFFATIPGADAETVKKKAKEFLDYINAKLPGLLELEYEGFYKRGFFVTKKKYAVIDEEDKITTVGLEIVRVDWSEIAKETQARVLEAILKHGDVEEAVRIVKEVTEKLSKYEVPPEKLVIYEQITRDLKDYKATGPHVAVAKRLAARGIKIRPGTVISYIVLKGSGRIGDRAIPFDEFDPAKHRYDAEYYIENQVLPAVERILRAFGYRKEDLRYQKTRQVGLGAWLKPKT